European Patent Specification EP 2 931 026 B1, published May 7, 2025. Title: Solanum lycopersicum plants having non-transgenic alterations in the acs2 gene. Applicant: Nunhems B.V. The sequence listing filed with the application follows.

SEQUENCE LISTING (24 sequences)

SEQ ID NO: 1 - protein, 485 aa, Lycopersicon esculentum
MGFEIAKTNSILSKLATNEEHGENSPYFDGWKAYDSDPFHPLKNPNGVIQMGLAENQLCLDLIEDWIKRNPKGSICSEGIKSFKAIANFQDYHGLPEFRKAIAKFMEKTRGGRVRFDPERVVMAGGATGANETIIFCLADPGDAFLVPSPYYPAFNRDLRWRTGVQLIPIHCESSNNFKITSKAVKEAYENAQKSNIKVKGLILTNPSNPLGTTLDKDTLKSVLSFTNQHNIHLVCDEIYAATVFDTPQFVSIAEILDEQEMTYCNKDLVHIVYSLSKDMGLPGFRVGIIYSFNDDVVNCARKMSSFGLVSTQTQYFLAAMLSDEKFVDNFLRESAMRLGKRHKHFTNGLEVVGIKCLKNNAGLFCWMDLRPLLRESTFDSEMSLWRVIINDVKLNVSPGSSFECQEPGWFRVCFANMDDGTVDIALARIRRFVGVEKSGDKSSSMEQKQQWKKNNLRLSFSKRMYDESVLSPLSSPIPPSPLVR

SEQ ID NO: 2 - protein, 485 aa, Lycopersicon esculentum
MGFEIAKTNSILSKLATNEEHGENSPYFDGWKAYDSDPFHPLKNPNGVIQMGLAENQLCLDLIEDWIKRNPKGSICSEGIKSFKAIANFQDYHGLPEFRKAITKFMEKTRGGRVRFDPERVVMAGGATGANETIIFCLADPGDAFLVPSPYYPAFNRDLRWRTGVQLIPIHCESSNNFKITSKAVKEAYENAQKSNIKVKGLILTNPSNPLGTTLDKDTLKSVLSFTNQHNIHLVCDEIYAATVFDTPQFVSIAEILDEQEMTYCNKDLVHIVYSLSKDMGLPGFRVGIIYSFNDDVVNCARKMSSFGLVSTQTQYFLAAMLSDEKFVDNFLRESAMRLGKRHKHFTNGLEVVGIKCLKNNAGLFCWMDLRPLLRESTFDSEMSLWRVIINDVKLNVSPGSSFECQEPGWFRVCFANMDDGTVDIALARIRRFVGVEKSGDKSSSMEQKQQWKKNNLRLSFSKRMYDESVLSPLSSPIPPSPLVR

SEQ ID NO: 3 - protein, 485 aa, Lycopersicon esculentum
MGFEIAKTNSILSKLATNEEHGENSPYFDGWKAYDSDPFHPLKNPNGVIQMGLAENQLCLDLIEDWIKRNPKGSICSEGIKSFKAIANFQDYHGLPEFRKAIAKFMEKTRGRRVRFDPERVVMAGGATGANETIIFCLADPGDAFLVPSPYYPAFNRDLRWRTGVQLIPIHCESSNNFKITSKAVKEAYENAQKSNIKVKGLILTNPSNPLGTTLDKDTLKSVLSFTNQHNIHLVCDEIYAATVFDTPQFVSIAEILDEQEMTYCNKDLVHIVYSLSKDMGLPGFRVGIIYSFNDDVVNCARKMSSFGLVSTQTQYFLAAMLSDEKFVDNFLRESAMRLGKRHKHFTNGLEVVGIKCLKNNAGLFCWMDLRPLLRESTFDSEMSLWRVIINDVKLNVSPGSSFECQEPGWFRVCFANMDDGTVDIALARIRRFVGVEKSGDKSSSMEQKQQWKKNNLRLSFSKRMYDESVLSPLSSPIPPSPLVR

SEQ ID NO: 4 - protein, 485 aa, Lycopersicon esculentum
MGFEIAKTNSILSKLATNEEHGENSPYFDGWKAYDSDPFHPLKNPNGVIQMGLAENQLCLDLIEDWIKRNPKGSICSEGIKSFKAIANFQDYHGLPEFRKAIAKFMEKTRGGRVRFDLERVVMAGGATGANETIIFCLADPGDAFLVPSPYYPAFNRDLRWRTGVQLIPIHCESSNNFKITSKAVKEAYENAQKSNIKVKGLILTNPSNPLGTTLDKDTLKSVLSFTNQHNIHLVCDEIYAATVFDTPQFVSIAEILDEQEMTYCNKDLVHIVYSLSKDMGLPGFRVGIIYSFNDDVVNCARKMSSFGLVSTQTQYFLAAMLSDEKFVDNFLRESAMRLGKRHKHFTNGLEVVGIKCLKNNAGLFCWMDLRPLLRESTFDSEMSLWRVIINDVKLNVSPGSSFECQEPGWFRVCFANMDDGTVDIALARIRRFVGVEKSGDKSSSMEQKQQWKKNNLRLSFSKRMYDESVLSPLSSPIPPSPLVR

SEQ ID NO: 5 - protein, 485 aa, Lycopersicon esculentum
MGFEIAKTNSILSKLATNEEHGENSPYFDGWKAYDSDPFHPLKNPNGVIQMGLAENQLCLDLIEDWIKRNPKGSICSEGIKSFKAIANFQDYHGLPEFRKVIAKFMEKTRGGRVRFDPERVVMAGGATGANETIIFCLADPGDAFLVPSPYYPAFNRDLRWRTGVQLIPIHCESSNNFKITSKAVKEAYENAQKSNIKVKGLILTNPSNPLGTTLDKDTLKSVLSFTNQHNIHLVCDEIYAATVFDTPQFVSIAEILDEQEMTYCNKDLVHIVYSLSKDMGLPGFRVGIIYSFNDDVVNCARKMSSFGLVSTQTQYFLAAMLSDEKFVDNFLRESAMRLGKRHKHFTNGLEVVGIKCLKNNAGLFCWMDLRPLLRESTFDSEMSLWRVIINDVKLNVSPGSSFECQEPGWFRVCFANMDDGTVDIALARIRRFVGVEKSGDKSSSMEQKQQWKKNNLRLSFSKRMYDESVLSPLSSPIPPSPLVR

SEQ ID NO: 6 - protein, 485 aa, Lycopersicon esculentum
MGFEIAKTNSILSKLATNEEHGENSPYFDGWKAYDSDPFHPLKNPNGVIQMGLAENQLCLDLIEDWIKRNPKGSICSEGIKSFKAIANFQDYHGLPEFRKTIAKFMEKTRGGRVRFDPERVVMAGGATGANETIIFCLADPGDAFLVPSPYYPAFNRDLRWRTGVQLIPIHCESSNNFKITSKAVKEAYENAQKSNIKVKGLILTNPSNPLGTTLDKDTLKSVLSFTNQHNIHLVCDEIYAATVFDTPQFVSIAEILDEQEMTYCNKDLVHIVYSLSKDMGLPGFRVGIIYSFNDDVVNCARKMSSFGLVSTQTQYFLAAMLSDEKFVDNFLRESAMRLGKRHKHFTNGLEVVGIKCLKNNAGLFCWMDLRPLLRESTFDSEMSLWRVIINDVKLNVSPGSSFECQEPGWFRVCFANMDDGTVDIALARIRRFVGVEKSGDKSSSMEQKQQWKKNNLRLSFSKRMYDESVLSPLSSPIPPSPLVR

SEQ ID NO: 7 - protein, 485 aa, Lycopersicon esculentum
MGFEIAKTNSILSKLATNEEHGENSPYFDGWKAYDSDPFHPLKNPNGVIQMGLAENQLCLDLIEDWIKRNPKGSICSEGIKSFKAIANFQDYHGLPEFRKAIAKFMEKTRGGRVRFDPERVVMAGGATGANETIIFCLADPGDAFLVPSPYYPAFNRDLRWRTGVQLIPIHCESSNNFKITSKAVKEAYENAQKSNIKVKGLILTNPSNPLGTTLDKDTLKSVLSFTNQHNIHLVCDEIYAATVFDTPQFVSIAEILDEQEMTYYNKDLVHIVYSLSKDMGLPGFRVGIIYSFNDDVVNCARKMSSFGLVSTQTQYFLAAMLSDEKFVDNFLRESAMRLGKRHKHFTNGLEVVGIKCLKNNAGLFCWMDLRPLLRESTFDSEMSLWRVIINDVKLNVSPGSSFECQEPGWFRVCFANMDDGTVDIALARIRRFVGVEKSGDKSSSMEQKQQWKKNNLRLSFSKRMYDESVLSPLSSPIPPSPLVR

SEQ ID NO: 8 - protein, 485 aa, Lycopersicon esculentum
MGFEIAKTNSILSKLATNEEHGENSPYFDGWKAYDSDPFHPLKNPNGVIQMGLAENQLCLDLIEDWIKRNPKGSICSEGIKSFKAIANFQDYHGLPEFRKAIAKFMEKTRGGRVRFDPERVVMAGGATGANETIIFCLADPGDAFLEPSPYYPAFNRDLRWRTGVQLIPIHCESSNNFKITSKAVKEAYENAQKSNIKVKGLILTNPSNPLGTTLDKDTLKSVLSFTNQHNIHLVCDEIYAATVFDTPQFVSIAEILDEQEMTYCNKDLVHIVYSLSKDMGLPGFRVGIIYSFNDDVVNCARKMSSFGLVSTQTQYFLAAMLSDEKFVDNFLRESAMRLGKRHKHFTNGLEVVGIKCLKNNAGLFCWMDLRPLLRESTFDSEMSLWRVIINDVKLNVSPGSSFECQEPGWFRVCFANMDDGTVDIALARIRRFVGVEKSGDKSSSMEQKQQWKKNNLRLSFSKRMYDESVLSPLSSPIPPSPLVR

SEQ ID NO: 9 - DNA, 1459 bp, Lycopersicon esculentum
atgggatttgagattgcaaagaccaactcaatcttatcaaaattggctactaatgaagagcatggcgaaaactcgccatattttgatgggtggaaagcatacgatagtgatcctttccaccctctaaaaaaccccaacggagttatccaaatgggtcttgctgaaaatcagctttgtttagacttgatagaagattggattaagagaaacccaaaaggttcaatttgttctgaaggaatcaaatcattcaaggccattgccaactttcaagattatcatggcttgcctgaattcagaaaagcgattgcgaaatttatggagaaaacaagaggaggaagagttagatttgatccagaaagagttgttatggctggtggtgccactggggctaatgagacaattatattttgtttggctgatcctggcgatgcatttttagtaccttcaccatactacccagcatttaacagagatttaagatggagaactggagtacaacttattccaattcactgtgagagctccaataatttcaaaattacttcaaaagcagtaaaagaagcatatgaaaatgcacaaaaatcaaacatcaaagtaaaaggtttgattttgaccaatccatcaaatccattgggcaccactttggacaaagacacactgaaaagtgtcttgagtttcaccaaccaacacaacatccaccttgtttgtgacgaaatctacgcagccactgtctttgacacgcctcaattcgtcagtatagctgaaatcctcgatgaacaggaaatgacttactgcaacaaagatttagttcacatcgtctacagtctttcaaaagacatggggttaccaggatttagagtcggaatcatatattcttttaacgacgatgtcgttaattgtgctagaaaaatgtcgagtttcggtttagtatctacacaaacgcaatattttttagcggcaatgctatcggacgaaaaattcgtcgataattttctaagagaaagcgcgatgaggttaggtaaaaggcacaaacattttactaatggacttgaagtagtgggaattaaatgcttgaaaaataatgcggggcttttttgttggatggatttgcgtccacttttaagggaatcgactttcgatagcgaaatgtcgttatggagagttattataaacgatgttaagcttaacgtctcgcctggatcttcgtttgaatgtcaagagccagggtggttccgagtttgttttgcaaatatggatgatggaacggttgatattgcgctcgcgaggattcggaggttcgtaggtgttgagaaaagtggagataaatcgagttcgatggaacagaagcaacaatggaagaagaataatttgagacttagtttttcgaaaagaatgtatgatgaaagtgttttgtcaccactttcgtcacctattcctccctcaccattagttcgttaag

SEQ ID NO: 10 - DNA, 1459 bp, Lycopersicon esculentum
atgggatttgagattgcaaagaccaactcaatcttatcaaaattggctactaatgaagagcatggcgaaaactcgccatattttgatgggtggaaagcatacgatagtgatcctttccaccctctaaaaaaccccaacggagttatccaaatgggtcttgctgaaaatcagctttgtttagacttgatagaagattggattaagagaaacccaaaaggttcaatttgttctgaaggaatcaaatcattcaaggccattgccaactttcaagattatcatggcttgcctgaattcagaaaagcgattacgaaatttatggagaaaacaagaggaggaagagttagatttgatccagaaagagttgttatggctggtggtgccactggggctaatgagacaattatattttgtttggctgatcctggcgatgcatttttagtaccttcaccatactacccagcatttaacagagatttaagatggagaactggagtacaacttattccaattcactgtgagagctccaataatttcaaaattacttcaaaagcagtaaaagaagcatatgaaaatgcacaaaaatcaaacatcaaagtaaaaggtttgattttgaccaatccatcaaatccattgggcaccactttggacaaagacacactgaaaagtgtcttgagtttcaccaaccaacacaacatccaccttgtttgtgacgaaatctacgcagccactgtctttgacacgcctcaattcgtcagtatagctgaaatcctcgatgaacaggaaatgacttactgcaacaaagatttagttcacatcgtctacagtctttcaaaagacatggggttaccaggatttagagtcggaatcatatattcttttaacgacgatgtcgttaattgtgctagaaaaatgtcgagtttcggtttagtatctacacaaacgcaatattttttagcggcaatgctatcggacgaaaaattcgtcgataattttctaagagaaagcgcgatgaggttaggtaaaaggcacaaacattttactaatggacttgaagtagtgggaattaaatgcttgaaaaataatgcggggcttttttgttggatggatttgcgtccacttttaagggaatcgactttcgatagcgaaatgtcgttatggagagttattataaacgatgttaagcttaacgtctcgcctggatcttcgtttgaatgtcaagagccagggtggttccgagtttgttttgcaaatatggatgatggaacggttgatattgcgctcgcgaggattcggaggttcgtaggtgttgagaaaagtggagataaatcgagttcgatggaacagaagcaacaatggaagaagaataatttgagacttagtttttcgaaaagaatgtatgatgaaagtgttttgtcaccactttcgtcacctattcctccctcaccattagttcgttaag

SEQ ID NO: 11 - DNA, 1459 bp, Lycopersicon esculentum
atgggatttgagattgcaaagaccaactcaatcttatcaaaattggctactaatgaagagcatggcgaaaactcgccatattttgatgggtggaaagcatacgatagtgatcctttccaccctctaaaaaaccccaacggagttatccaaatgggtcttgctgaaaatcagctttgtttagacttgatagaagattggattaagagaaacccaaaaggttcaatttgttctgaaggaatcaaatcattcaaggccattgccaactttcaagattatcatggcttgcctgaattcagaaaagcgattgcgaaatttatggagaaaacaagaggaagaagagttagatttgatccagaaagagttgttatggctggtggtgccactggggctaatgagacaattatattttgtttggctgatcctggcgatgcatttttagtaccttcaccatactacccagcatttaacagagatttaagatggagaactggagtacaacttattccaattcactgtgagagctccaataatttcaaaattacttcaaaagcagtaaaagaagcatatgaaaatgcacaaaaatcaaacatcaaagtaaaaggtttgattttgaccaatccatcaaatccattgggcaccactttggacaaagacacactgaaaagtgtcttgagtttcaccaaccaacacaacatccaccttgtttgtgacgaaatctacgcagccactgtctttgacacgcctcaattcgtcagtatagctgaaatcctcgatgaacaggaaatgacttactgcaacaaagatttagttcacatcgtctacagtctttcaaaagacatggggttaccaggatttagagtcggaatcatatattcttttaacgacgatgtcgttaattgtgctagaaaaatgtcgagtttcggtttagtatctacacaaacgcaatattttttagcggcaatgctatcggacgaaaaattcgtcgataattttctaagagaaagcgcgatgaggttaggtaaaaggcacaaacattttactaatggacttgaagtagtgggaattaaatgcttgaaaaataatgcggggcttttttgttggatggatttgcgtccacttttaagggaatcgactttcgatagcgaaatgtcgttatggagagttattataaacgatgttaagcttaacgtctcgcctggatcttcgtttgaatgtcaagagccagggtggttccgagtttgttttgcaaatatggatgatggaacggttgatattgcgctcgcgaggattcggaggttcgtaggtgttgagaaaagtggagataaatcgagttcgatggaacagaagcaacaatggaagaagaataatttgagacttagtttttcgaaaagaatgtatgatgaaagtgttttgtcaccactttcgtcacctattcctccctcaccattagttcgttaag

SEQ ID NO: 12 - DNA, 1459 bp, Lycopersicon esculentum
atgggatttgagattgcaaagaccaactcaatcttatcaaaattggctactaatgaagagcatggcgaaaactcgccatattttgatgggtggaaagcatacgatagtgatcctttccaccctctaaaaaaccccaacggagttatccaaatgggtcttgctgaaaatcagctttgtttagacttgatagaagattggattaagagaaacccaaaaggttcaatttgttctgaaggaatcaaatcattcaaggccattgccaactttcaagattatcatggcttgcctgaattcagaaaagcgattgcgaaatttatggagaaaacaagaggaggaagagttagatttgatctagaaagagttgttatggctggtggtgccactggggctaatgagacaattatattttgtttggctgatcctggcgatgcatttttagtaccttcaccatactacccagcatttaacagagatttaagatggagaactggagtacaacttattccaattcactgtgagagctccaataatttcaaaattacttcaaaagcagtaaaagaagcatatgaaaatgcacaaaaatcaaacatcaaagtaaaaggtttgattttgaccaatccatcaaatccattgggcaccactttggacaaagacacactgaaaagtgtcttgagtttcaccaaccaacacaacatccaccttgtttgtgacgaaatctacgcagccactgtctttgacacgcctcaattcgtcagtatagctgaaatcctcgatgaacaggaaatgacttactgcaacaaagatttagttcacatcgtctacagtctttcaaaagacatggggttaccaggatttagagtcggaatcatatattcttttaacgacgatgtcgttaattgtgctagaaaaatgtcgagtttcggtttagtatctacacaaacgcaatattttttagcggcaatgctatcggacgaaaaattcgtcgataattttctaagagaaagcgcgatgaggttaggtaaaaggcacaaacattttactaatggacttgaagtagtgggaattaaatgcttgaaaaataatgcggggcttttttgttggatggatttgcgtccacttttaagggaatcgactttcgatagcgaaatgtcgttatggagagttattataaacgatgttaagcttaacgtctcgcctggatcttcgtttgaatgtcaagagccagggtggttccgagtttgttttgcaaatatggatgatggaacggttgatattgcgctcgcgaggattcggaggttcgtaggtgttgagaaaagtggagataaatcgagttcgatggaacagaagcaacaatggaagaagaataatttgagacttagtttttcgaaaagaatgtatgatgaaagtgttttgtcaccactttcgtcacctattcctccctcaccattagttcgttaag

SEQ ID NO: 13 - DNA, 1459 bp, Lycopersicon esculentum
atgggatttgagattgcaaagaccaactcaatcttatcaaaattggctactaatgaagagcatggcgaaaactcgccatattttgatgggtggaaagcatacgatagtgatcctttccaccctctaaaaaaccccaacggagttatccaaatgggtcttgctgaaaatcagctttgtttagacttgatagaagattggattaagagaaacccaaaaggttcaatttgttctgaaggaatcaaatcattcaaggccattgccaactttcaagattatcatggcttgcctgaattcagaaaagtgattgcgaaatttatggagaaaacaagaggaggaagagttagatttgatccagaaagagttgttatggctggtggtgccactggggctaatgagacaattatattttgtttggctgatcctggcgatgcatttttagtaccttcaccatactacccagcatttaacagagatttaagatggagaactggagtacaacttattccaattcactgtgagagctccaataatttcaaaattacttcaaaagcagtaaaagaagcatatgaaaatgcacaaaaatcaaacatcaaagtaaaaggtttgattttgaccaatccatcaaatccattgggcaccactttggacaaagacacactgaaaagtgtcttgagtttcaccaaccaacacaacatccaccttgtttgtgacgaaatctacgcagccactgtctttgacacgcctcaattcgtcagtatagctgaaatcctcgatgaacaggaaatgacttactgcaacaaagatttagttcacatcgtctacagtctttcaaaagacatggggttaccaggatttagagtcggaatcatatattcttttaacgacgatgtcgttaattgtgctagaaaaatgtcgagtttcggtttagtatctacacaaacgcaatattttttagcggcaatgctatcggacgaaaaattcgtcgataattttctaagagaaagcgcgatgaggttaggtaaaaggcacaaacattttactaatggacttgaagtagtgggaattaaatgcttgaaaaataatgcggggcttttttgttggatggatttgcgtccacttttaagggaatcgactttcgatagcgaaatgtcgttatggagagttattataaacgatgttaagcttaacgtctcgcctggatcttcgtttgaatgtcaagagccagggtggttccgagtttgttttgcaaatatggatgatggaacggttgatattgcgctcgcgaggattcggaggttcgtaggtgttgagaaaagtggagataaatcgagttcgatggaacagaagcaacaatggaagaagaataatttgagacttagtttttcgaaaagaatgtatgatgaaagtgttttgtcaccactttcgtcacctattcctccctcaccattagttcgttaag

SEQ ID NO: 14 - DNA, 1459 bp, Lycopersicon esculentum
atgggatttgagattgcaaagaccaactcaatcttatcaaaattggctactaatgaagagcatggcgaaaactcgccatattttgatgggtggaaagcatacgatagtgatcctttccaccctctaaaaaaccccaacggagttatccaaatgggtcttgctgaaaatcagctttgtttagacttgatagaagattggattaagagaaacccaaaaggttcaatttgttctgaaggaatcaaatcattcaaggccattgccaactttcaagattatcatggcttgcctgaattcagaaaaacgattgcgaaatttatggagaaaacaagaggaggaagagttagatttgatccagaaagagttgttatggctggtggtgccactggggctaatgagacaattatattttgtttggctgatcctggcgatgcatttttagtaccttcaccatactacccagcatttaacagagatttaagatggagaactggagtacaacttattccaattcactgtgagagctccaataatttcaaaattacttcaaaagcagtaaaagaagcatatgaaaatgcacaaaaatcaaacatcaaagtaaaaggtttgattttgaccaatccatcaaatccattgggcaccactttggacaaagacacactgaaaagtgtcttgagtttcaccaaccaacacaacatccaccttgtttgtgacgaaatctacgcagccactgtctttgacacgcctcaattcgtcagtatagctgaaatcctcgatgaacaggaaatgacttactgcaacaaagatttagttcacatcgtctacagtctttcaaaagacatggggttaccaggatttagagtcggaatcatatattcttttaacgacgatgtcgttaattgtgctagaaaaatgtcgagtttcggtttagtatctacacaaacgcaatattttttagcggcaatgctatcggacgaaaaattcgtcgataattttctaagagaaagcgcgatgaggttaggtaaaaggcacaaacattttactaatggacttgaagtagtgggaattaaatgcttgaaaaataatgcggggcttttttgttggatggatttgcgtccacttttaagggaatcgactttcgatagcgaaatgtcgttatggagagttattataaacgatgttaagcttaacgtctcgcctggatcttcgtttgaatgtcaagagccagggtggttccgagtttgttttgcaaatatggatgatggaacggttgatattgcgctcgcgaggattcggaggttcgtaggtgttgagaaaagtggagataaatcgagttcgatggaacagaagcaacaatggaagaagaataatttgagacttagtttttcgaaaagaatgtatgatgaaagtgttttgtcaccactttcgtcacctattcctccctcaccattagttcgttaag

SEQ ID NO: 15 - DNA, 1459 bp, Lycopersicon esculentum
atgggatttgagattgcaaagaccaactcaatcttatcaaaattggctactaatgaagagcatggcgaaaactcgccatattttgatgggtggaaagcatacgatagtgatcctttccaccctctaaaaaaccccaacggagttatccaaatgggtcttgctgaaaatcagctttgtttagacttgatagaagattggattaagagaaacccaaaaggttcaatttgttctgaaggaatcaaatcattcaaggccattgccaactttcaagattatcatggcttgcctgaattcagaaaagcgattgcgaaatttatggagaaaacaagaggaggaagagttagatttgatccagaaagagttgttatggctggtggtgccactggggctaatgagacaattatattttgtttggctgatcctggcgatgcatttttagtaccttcaccatactacccagcatttaacagagatttaagatggagaactggagtacaacttattccaattcactgtgagagctccaataatttcaaaattacttcaaaagcagtaaaagaagcatatgaaaatgcacaaaaatcaaacatcaaagtaaaaggtttgattttgaccaatccatcaaatccattgggcaccactttggacaaagacacactgaaaagtgtcttgagtttcaccaaccaacacaacatccaccttgtttgtgacgaaatctacgcagccactgtctttgacacgcctcaattcgtcagtatagctgaaatcctcgatgaacaggaaatgacttactacaacaaagatttagttcacatcgtctacagtctttcaaaagacatggggttaccaggatttagagtcggaatcatatattcttttaacgacgatgtcgttaattgtgctagaaaaatgtcgagtttcggtttagtatctacacaaacgcaatattttttagcggcaatgctatcggacgaaaaattcgtcgataattttctaagagaaagcgcgatgaggttaggtaaaaggcacaaacattttactaatggacttgaagtagtgggaattaaatgcttgaaaaataatgcggggcttttttgttggatggatttgcgtccacttttaagggaatcgactttcgatagcgaaatgtcgttatggagagttattataaacgatgttaagcttaacgtctcgcctggatcttcgtttgaatgtcaagagccagggtggttccgagtttgttttgcaaatatggatgatggaacggttgatattgcgctcgcgaggattcggaggttcgtaggtgttgagaaaagtggagataaatcgagttcgatggaacagaagcaacaatggaagaagaataatttgagacttagtttttcgaaaagaatgtatgatgaaagtgttttgtcaccactttcgtcacctattcctccctcaccattagttcgttaag

SEQ ID NO: 16 - DNA, 1459 bp, Lycopersicon esculentum
atgggatttgagattgcaaagaccaactcaatcttatcaaaattggctactaatgaagagcatggcgaaaactcgccatattttgatgggtggaaagcatacgatagtgatcctttccaccctctaaaaaaccccaacggagttatccaaatgggtcttgctgaaaatcagctttgtttagacttgatagaagattggattaagagaaacccaaaaggttcaatttgttctgaaggaatcaaatcattcaaggccattgccaactttcaagattatcatggcttgcctgaattcagaaaagcgattgcgaaatttatggagaaaacaagaggaggaagagttagatttgatccagaaagagttgttatggctggtggtgccactggggctaatgagacaattatattttgtttggctgatcctggcgatgcatttttagaaccttcaccatactacccagcatttaacagagatttaagatggagaactggagtacaacttattccaattcactgtgagagctccaataatttcaaaattacttcaaaagcagtaaaagaagcatatgaaaatgcacaaaaatcaaacatcaaagtaaaaggtttgattttgaccaatccatcaaatccattgggcaccactttggacaaagacacactgaaaagtgtcttgagtttcaccaaccaacacaacatccaccttgtttgtgacgaaatctacgcagccactgtctttgacacgcctcaattcgtcagtatagctgaaatcctcgatgaacaggaaatgacttactgcaacaaagatttagttcacatcgtctacagtctttcaaaagacatggggttaccaggatttagagtcggaatcatatattcttttaacgacgatgtcgttaattgtgctagaaaaatgtcgagtttcggtttagtatctacacaaacgcaatattttttagcggcaatgctatcggacgaaaaattcgtcgataattttctaagagaaagcgcgatgaggttaggtaaaaggcacaaacattttactaatggacttgaagtagtgggaattaaatgcttgaaaaataatgcggggcttttttgttggatggatttgcgtccacttttaagggaatcgactttcgatagcgaaatgtcgttatggagagttattataaacgatgttaagcttaacgtctcgcctggatcttcgtttgaatgtcaagagccagggtggttccgagtttgttttgcaaatatggatgatggaacggttgatattgcgctcgcgaggattcggaggttcgtaggtgttgagaaaagtggagataaatcgagttcgatggaacagaagcaacaatggaagaagaataatttgagacttagtttttcgaaaagaatgtatgatgaaagtgttttgtcaccactttcgtcacctattcctccctcaccattagttcgttaag

SEQ ID NO: 17 - DNA, 2523 bp, Lycopersicon esculentum
  exon (1)..(171): Exon 1
  exon (270)..(399): Exon 2
  exon (485)..(644): Exon 3
  exon (1526)..(2523): Exon 4
atgggatttgagattgcaaagaccaactcaatcttatcaaaattggctactaatgaagagcatggcgaaaactcgccatattttgatgggtggaaagcatacgatagtgatcctttccaccctctaaaaaaccccaacggagttatccaaatgggtcttgctgaaaatcaggtaattaattatcctttatttatatattttgcagtttgaccaaacagactattataatttttttctgaaacctcgatggtgttaaatttcttttgtagctttgtttagacttgatagaagattggattaagagaaacccaaaaggttcaatttgttctgaaggaatcaaatcattcaaggccattgccaactttcaagattatcatggcttgcctgaattcagaaaagtacatatcgtactatagtcagttaaattatattgatagtataaaaattcgttaatatatttaactaacgagtttatttaatcaggcgattgcgaaatttatggagaaaacaagaggaggaagagttagatttgatccagaaagagttgttatggctggtggtgccactggagctaatgagacaattatattttgtttggctgatcctggcgatgcatttttagtaccttcaccatactacccagcgtaagtatatttaattatatatgtgtaaaaaaaattaaaatcatcaaatcattttttttatttgtattaccaaataaattgtctaattttcaagattgtaacacattcatcaaagtacctaataatataaacgattcagtatattaacgatgtatataatttaattcctttggcggatttgtctttttatgttgggccatcagaagaacattctggtgtattaattaattaattaattaataatagatgtgttgtcattcttttttaagacagcgagagtttaattagtcttaattactggattatcacgcaagctctttcttgaattttattattcttatattaaacacatgatagcataatatctttcttttgtggaatccagcttgttcgtgaagctttgtattcacacttataaaacaacaaaaaataaaatctggtggtaattgattaaagagagaaatataaaaaaataatagtcaaatagactaataaggaaagaaataaaaaatacacaaaatactaaaaaaaaagaattaaggtatagtggtctattattgagaacttttttgaagaattgaaccccactttaatttcttgcttgacccgtgaccattgcttatcgaggtaaaataaaatttcaaacattgactatgacttgttagagagtaattaccacaagtcaaaattttgttactctgtctcgttatttcattaggatcgataagataacatctaacatatatatcttttttattagtacttgtttatttttagtaaaagcacgttatacattttacaatagtcaattgttgcatatattagtatatatattttgctaagtcctaactaacaatatttttggcaattgactaatgcagatttaacagagatttaagatggagaactggagtacaacttattccaattcactgtgagagctccaataatttcaaaattacttcaaaagcagtaaaagaagcatatgaaaatgcacaaaaatcaaacatcaaagtaaaaggtttgattttgaccaatccatcaaatccattgggcaccactttggacaaagacacactgaaaagtgtcttgagtttcaccaaccaacacaacatccaccttgtttgtgacgaaatctacgcagccactgtctttgacacgcctcaattcgtcagtatagctgaaatcctcgatgaacaggaaatgacttactgcaacaaagatttagttcacatcgtctacagtctttcaaaagacatggggttaccaggatttagagtcggaatcatatattcttttaacgacgatgtcgttaattgtgctagaaaaatgtcgagtttcggtttagtatctacacaaacgcaatattttttagcggcaatgctatcggacgaaaaattcgtcgataattttctaagagaaagcgcgatgaggttaggtaaaaggcacaaacattttactaatggacttgaagtagtgggaattaaatgcttgaaaaataatgcggggcttttttgttggatggatttgcgtccacttttaagggaatcgactttcgatagcgaaatgtcgttatggagagttattataaacgatgttaagcttaacgtctcgcctggatcttcgtttgaatgtcaagagccagggtggttccgagtttgttttgcaaatatggatgatggaacggttgatattgcgctcgcgaggattcggaggttcgtaggtgttgagaaaagtggagataaatcgagttcgatggaaaagaagcaacaatggaagaagaataatttgagacttagtttttcgaaaagaatgtatgatgaaagtgttttgtcaccactttcgtcacctattcctccctcaccattagttcgttaag

SEQ ID NO: 18 - protein, 97 aa, Lycopersicon esculentum
LCLDLIEDWIKRNPKGSICSEGIKSFKAIANFQDYHGLPEFRKAITKFMEKTRGGRVRFDPERVVMAGGATGANETIIFCLADPGDAFLVPSPYYPA

SEQ ID NO: 19 - protein, 97 aa, Lycopersicon esculentum
LCLDLIEDWIKRNPKGSICSEGIKSFKAIANFQDYHGLPEFRKAIAKFMEKTRGRRVRFDPERVVMAGGATGANETIIFCLADPGDAFLVPSPYYPA

SEQ ID NO: 20 - protein, 97 aa, Lycopersicon esculentum
LCLDLIEDWIKRNPKGSICSEGIKSFKAIANFQDYHGLPEFRKAIAKFMEKTRGGRVRFDLERVVMAGGATGANETIIFCLADPGDAFLVPSPYYPA

SEQ ID NO: 21 - protein, 97 aa, Lycopersicon esculentum
LCLDLIEDWIKRNPKGSICSEGIKSFKAIANFQDYHGLPEFRKVIAKFMEKTRGGRVRFDPERVVMAGGATGANETIIFCLADPGDAFLVPSPYYPA

SEQ ID NO: 22 - protein, 97 aa, Lycopersicon esculentum
LCLDLIEDWIKRNPKGSICSEGIKSFKAIANFQDYHGLPEFRKTIAKFMEKTRGGRVRFDPERVVMAGGATGANETIIFCLADPGDAFLVPSPYYPA

SEQ ID NO: 23 - protein, 115 aa, Lycopersicon esculentum
  misc_feature (115)..(115): Xaa can be any naturally occurring amino acid
AVKEAYENAQKSNIKVKGLILTNPSNPLGTTLDKDTLKSVLSFTNQHNIHLVCDEIYAATVFDTPQFVSIAEILDEQEMTYYNKDLVHIVYSLSKDMGLPGFRVGIIYSFNDDVX

SEQ ID NO: 24 - protein, 97 aa, Lycopersicon esculentum
LCLDLIEDWIKRNPKGSICSEGIKSFKAIANFQDYHGLPEFRKAIAKFMEKTRGGRVRFDPERVVMAGGATGANETIIFCLADPGDAFLEPSPYYPA